European Patent Application EP 4 173 636 A1, published May 3, 2023. Title: Combination of anti-CCR8 antibody and chemotherapeutic agents. Applicant: SHIONOGI & CO., LTD. The sequence listing filed with the application follows.

SEQUENCE LISTING (60 sequences)

SEQ ID NO: 1 - protein, 355 aa, Homo sapiens
MDYTLDLSVTTVTDYYYPDIFSSPCDAELIQTNGKLLLAVFYCLLFVFSLLGNSLVILVLVVCKKLRSITDVYLLNLALSDLLFVFSFPFQTYYLLDQWVFGTVMCKVVSGFYYIGFYSSMFFITLMSVDRYLAVVHAVYALKVRTIRMGTTLCLAVWLTAIMATIPLLVFYQVASEDGVLQCYSFYNQQTLKWKIFTNFKMNILGLLIPFTIFMFCYIKILHQLKRCQNHNKTKAIRLVLIVVIASLLFWVPFNVVLFLTSLHSMHILDGCSISQQLTYATHVTEIISFTHCCVNPVIYAFVGEKFKKHLSEIFQKSCSQIFNYLGRQMPRESCEKSSSCQQHSSRSSSVDYIL

SEQ ID NO: 2 - protein, 16 aa, Artificial Sequence
  CDR1 of 10A11 VL
RSSKSLLHSNGNTYLY

SEQ ID NO: 3 - protein, 7 aa, Artificial Sequence
  CDR2 of 10A11 VL
RMSNLAS

SEQ ID NO: 4 - protein, 9 aa, Artificial Sequence
  CDR3 of 10A11 VL
MQHLEYPLT

SEQ ID NO: 5 - protein, 5 aa, Artificial Sequence
  CDR1 of 10A11 VH
TYALY

SEQ ID NO: 6 - protein, 19 aa, Artificial Sequence
  CDR2 of 10A11 VH
RIRSKSNNYATYYADSVKD

SEQ ID NO: 7 - protein, 14 aa, Artificial Sequence
  CDR3 of 10A11 VH
ARFYYSDYGYAMDY

SEQ ID NO: 8 - protein, 5 aa, Artificial Sequence
  CDR2 of 27G1 VH
TYAMY

SEQ ID NO: 9 - protein, 7 aa, Artificial Sequence
  CDR2 of 19D7 VL
RVSNLAS

SEQ ID NO: 10 - protein, 9 aa, Artificial Sequence
  CDR3 of 19D7 VL
MQHLEYPFT

SEQ ID NO: 11 - protein, 12 aa, Artificial Sequence
  CDR3 of 19D7 VH
GGYGNYRYAMDY

SEQ ID NO: 12 - protein, 5 aa, Artificial Sequence
  CDR1 of 8F7 VH
PYAMY

SEQ ID NO: 13 - protein, 8 aa, Artificial Sequence
  CDR3 of 8F7 VH
GHQGTMDY

SEQ ID NO: 14 - protein, 16 aa, Artificial Sequence
  CDR1 of 2C7 VL
RSSQSLVHSNGNTYLH

SEQ ID NO: 15 - protein, 7 aa, Artificial Sequence
  CDR2 of 2C7 VL
KVSNRFS

SEQ ID NO: 16 - protein, 9 aa, Artificial Sequence
  CDR3 of 2C7 VL
SQSTQVPLT

SEQ ID NO: 17 - protein, 5 aa, Artificial Sequence
  CDR1 of 2C7 VH
AYGVH

SEQ ID NO: 18 - protein, 16 aa, Artificial Sequence
  CDR2 of 2C7 VH
VIWRGGSTDYNAAFMS

SEQ ID NO: 19 - protein, 9 aa, Artificial Sequence
  CDR3 of 2C7 VH
KGGSYAMDY

SEQ ID NO: 20 - protein, 15 aa, Artificial Sequence
  CDR1 of 2-7B VL
RASQSVSISRYNIMH

SEQ ID NO: 21 - protein, 7 aa, Artificial Sequence
  CDR2 of 2-7B VL
RASNLAS

SEQ ID NO: 22 - protein, 9 aa, Artificial Sequence
  CDR3 of 2-7B VL
QQSRESPPT

SEQ ID NO: 23 - protein, 5 aa, Artificial Sequence
  CDR1 of 2-7B VH
DYYMA

SEQ ID NO: 24 - protein, 17 aa, Artificial Sequence
  CDR2 of 2-7B VH
TITYDVYSTYYRDSVKG

SEQ ID NO: 25 - protein, 14 aa, Artificial Sequence
  CDR3 of 2-7B VH
HGGDGYNSGNWFAY

SEQ ID NO: 26 - protein, 113 aa, Artificial Sequence
  10A11 VL
DIVMTQAAPSVPVTPGESVSISCRSSKSLLHSNGNTYLYWFLQRPGQSPQLLIYRMSNLASGVPDRFSGSGSGTAFTLRISRVEAEDVGVYYCMQHLEYPLTFGAGTKLELKR

SEQ ID NO: 27 - protein, 125 aa, Artificial Sequence
  10A11 VH
EVQLVESGGRLVQPKGSLKLSCAASGFAFNTYALYWIRQAPGKGLEWVARIRSKSNNYATYYADSVKDRFTISRDDSQSMLYLQMNNLKTEDTAMYYCVRARFYYSDYGYAMDYWGQGTSVTVSS

SEQ ID NO: 28 - protein, 125 aa, Artificial Sequence
  27G1 VH
EVQLVESGGRLVQPKGSLKLSCAASGFAFNTYAMYWIRQAPGKGLEWVARIRSKSNNYATYYADSVKDRFTISRDDSQSMLYLQMNNLKTEDTAMYYCVRARFYYSDYGYAMDYWGQGTSVTVSS

SEQ ID NO: 29 - protein, 113 aa, Artificial Sequence
  1H4 VL
DIVMTQAAPSVPVTPGESVSISCRSSKSLLHSNGNTYLYWFLQRPGQSPQLLIYRMSNLASGVPDRFSASGSGTAFTLRISRVEAEDVGVYYCMQHLEYPLTFGAGTKLELKR

SEQ ID NO: 30 - protein, 125 aa, Artificial Sequence
  1H4 VH
EVQLVESGGRLVQPKGSLKLSCAASGFTFNTYAMYWIRQAPGKGLEWVARIRSKSNNYATYYADSVKDRFTISRDDSQSMLYLQMNNLKTEDTAMYYCVRARFYYSDYGYAMDYWGQGTSVTVSS

SEQ ID NO: 31 - protein, 113 aa, Artificial Sequence
  19D7 VL
DIVMTQAAPSVPVTPGESVSISCRSSKSLLHSNGNTYLYWFLQRPGQSPQLLIYRVSNLASGVPDRFSGSGSGAAFTLRISRVEAEDVGVYYCMQHLEYPFTFGSGTKLEIKR

SEQ ID NO: 32 - protein, 123 aa, Artificial Sequence
  19D7 VH
EVQLVESGGRLVQPKGSLKLSCAASGFTFNTYAMYWIRQAPGKGLEWVARIRSKSNNYATYYADSVKDRFTISRDDSQSMLYLQMNNLKTEDTAMYYCVRGGYGNYRYAMDYWGQGTSVTVSS

SEQ ID NO: 33 - protein, 113 aa, Artificial Sequence
  8F7 VL
DIVMTQAAPSVPVTPGESVSISCRSSKSLLHSNGNTYLYWFLQRPGQSPQLLTYRMSNLASGVPDRFSGSGSGTAFTLRISRVEAEDVGVYYCMQHLEYPFTFGGGTKLEIKR

SEQ ID NO: 34 - protein, 119 aa, Artificial Sequence
  8F7 VH
EVQLVESGGRLVQPKRSLKLSCAASGFTFNPYAMYWIRQAPGQGLEWVARIRSKSNNYATYYADSVKDRFTISRDDSQSMLYLQMNNLKTEDTAMYYCVRGHQGTMDYWGQGTSVTVSS

SEQ ID NO: 35 - protein, 113 aa, Artificial Sequence
  2C7 VL
DVVLTQTPLSLPVSLGGQASISCRSSQSLVHSNGNTYLHWYLQKPGQSPKLLIYKVSNRFSGVPDRFSGSGSGTDFTLKISRVEAEDLGVYFCSQSTQVPLTFGAGTKLELKR

SEQ ID NO: 36 - protein, 117 aa, Artificial Sequence
  2C7 VH
QVQLKQSGPSLVQPSQSLSITCTVSGFSLTAYGVHWIRQSPGKGQEWLGVIWRGGSTDYNAAFMSRLTITKDNSKSQVFFKMNSLQADDTAIYYCAKKGGSYAMDYWGQGTSVTVSS

SEQ ID NO: 37 - protein, 111 aa, Artificial Sequence
  2-7B VL
DIVLTQSPALAVSLGQRATISCRASQSVSISRYNIMHWYQQKPGQQPKLLIYRASNLASGIPARFSGSGSGTDFTLTINPVQADDIATYYCQQSRESPPTFGGGTKLELKR

SEQ ID NO: 38 - protein, 123 aa, Artificial Sequence
  2-7B VH
EVQLVESDGGLVQPGRSLKLSCAASGFTFSDYYMAWVRQAPTKGLEWVATITYDVYSTYYRDSVKGRFTISRDNAKSTLYLQMDSLRSEDTATYYCARHGGDGYNSGNWFAYWGQGTLVTVSS

SEQ ID NO: 39 - protein, 353 aa, Mus musculus
MDYTMEPNVTMTDYYPDFFTAPCDAEFLLRGSMLYLAILYCVLFVLGLLGNSLVILVLVGCKKLRSITDIYLLNLAASDLLFVLSIPFQTHNLLDQWVFGTAMCKVVSGLYYIGFFSSMFFITLMSVDRYLAIVHAVYAIKVRTASVGTALSLTVWLAAVTATIPLMVFYQVASEDGMLQCFQFYEEQSLRWKLFTHFEINALGLLLPFAILLFCYVRILQQLRGCLNHNRTRAIKLVLTVVIVSLLFWVPFNVALFLTSLHDLHILDGCATRQRLALAIHVTEVISFTHCCVNPVIYAFIGEKFKKHLMDVFQKSCSHIFLYLGRQMPVGALERQLSSNQRSSHSSTLDDIL

SEQ ID NO: 40 - protein, 114 aa, Artificial Sequence
  10A11-IGKV3-20
EIVLTQSPGTLSLSPGERATLSCRSSKSLLHSNGNTYLYWYQQKPGQAPRLLIYRMSNLASGIPDRFSGSGSGTDFTLTISRLEPEDFAVYYCMQHLEYPLTFGQGTKVEIKRT

SEQ ID NO: 41 - protein, 125 aa, Artificial Sequence
  10A11-IGHV3-15 T94R
EVQLVESGGALVKPGGSLRLSCAASGFTFSTYALYWVRQAPGKGLEWVGRIRSKSNNYATYYADSVKDRFTISRDDSKNTLYLQMNSLKTEDTAVYYCTRARFYYSDYGYAMDYWGQGTLVTVSS

SEQ ID NO: 42 - protein, 114 aa, Artificial Sequence
  10A11-IGKV4-1
DIVMTQSPDSLAVSLGERATINCRSSKSLLHSNGNTYLYWYQQKPGQPPKLLIYRMSNLASGVPDRFSGSGSGTDFTLTISSLQAEDVAVYYCMQHLEYPLTFGQGTKLEIKRT

SEQ ID NO: 43 - protein, 114 aa, Artificial Sequence
  10A11-IGKV1-39
DIQMTQSPSSLSASVGDRVTITCRSSKSLLHSNGNTYLYWYQQKPGKAPKLLIYRMSNLASGVPSRFSGSGSGTDFTLTISSLQPEDFATYYCMQHLEYPLTFGQGTKLEIKRT

SEQ ID NO: 44 - protein, 114 aa, Artificial Sequence
  10A11-IGKV2-40
DIVMTQTPLSLPVTPGEPASISCRSSKSLLHSNGNTYLYWYLQKPGQSPQLLIYRMSNLASGVPDRFSGSGSGTDFTLKISRVEAEDVGVYYCMQHLEYPLTFGQGTKLEIKRT

SEQ ID NO: 45 - protein, 114 aa, Artificial Sequence
  10A11-IGKV1-16
DIQMTQSPSSLSASVGDRVTITCRSSKSLLHSNGNTYLYWFQQKPGKAPKSLIYRMSNLASGVPSRFSGSGSGTDFTLTISSLQPEDFATYYCMQHLEYPLTFGQGTKLEIKRT

SEQ ID NO: 46 - protein, 125 aa, Artificial Sequence
  10A11-IGHV3-73
EVQLVESGGGLVQPGGSLKLSCAASGFAFNTYALYWVRQASGKGLEWVGRIRSKSNNYATYYADSVKDRFTISRDDSKNTAYLQMNSLKTEDTAVYYCTRARFYYSDYGYAMDYWGQGTLVTVSS

SEQ ID NO: 47 - protein, 114 aa, Artificial Sequence
  10A11-IGKV2-28
DIVMTQSPLSLPVTPGEPASISCRSSKSLLHSNGNTYLYWYLQKPGQSPQLLIYRMSNLASGVPDRFSGSGSGTDFTLKISRVEAEDVGVYYCMQHLEYPLTFGQGTKVEIKRT

SEQ ID NO: 48 - protein, 360 aa, Homo sapiens
MNPTDIADTTLDESIYSNYYLYESIPKPCTKEGIKAFGELFLPPLYSLVFVFGLLGNSVVVLVLFKYKRLRSMTDVYLLNLAISDLLFVFSLPFWGYYAADQWVFGLGLCKMISWMYLVGFYSGIFFVMLMSIDRYLAIVHAVFSLRARTLTYGVITSLATWSVAVFASLPGFLFSTCYTERNHTYCKTKYSLNSTTWKVLSSLEINILGLVIPLGIMLFCYSMIIRTLQHCKNEKKNKAVKMIFAVVVLFLGFWTPYNIVLFLETLVELEVLQDCTFERYLDYAIQATETLAFVHCCLNPIIYFFLGEKFRKYILQLFKTCRGLFVLCQYCGLLQIYSADTPSSSYTQSTMDHDLHDAL

SEQ ID NO: 49 - protein, 7 aa, Artificial Sequence
  CDR2 consensus sequence of VL
  misc_feature (2)..(2): Xaa can be any naturally occurring amino acid
RXSNLAS

SEQ ID NO: 50 - protein, 9 aa, Artificial Sequence
  CDR3 consensus sequence of VL
  misc_feature (8)..(8): Xaa can be any naturally occurring amino acid
MQHLEYPXT

SEQ ID NO: 51 - protein, 5 aa, Artificial Sequence
  CDR1 consensus sequence of VH
  misc_feature (1)..(1): Xaa can be any naturally occurring amino acid
  misc_feature (4)..(4): Xaa can be any naturally occurring amino acid
XYAXY

SEQ ID NO: 52 - protein, 105 aa, Artificial Sequence [sequence omitted]

SEQ ID NO: 53 - protein, 329 aa, Artificial Sequence
  h10A11 CH
ASTKGPSVFPLAPSSKSTSGGTAALGCLVKDYFPEPVTVSWNSGALTSGVHTFPAVLQSSGLYSLSSVVTVPSSSLGTQTYICNVNHKPSNTKVDKRVEPKSCDKTHTCPPCPAPELLGGPSVFLFPPKPKDTLMISRTPEVTCVVVDVSHEDPEVKFNWYVDGVEVHNAKTKPREEQYNSTYRVVSVLTVLHQDWLNGKEYKCKVSNKALPAPIEKTISKAKGQPREPQVYTLPPSREEMTKNQVSLTCLVKGFYPSDIAVEWESNGQPENNYKTTPPVLDSDGSFFLYSKLTVDKSRWQQGNVFSCSVMHEALHNHYTQKSLSLSPG

SEQ ID NO: 54 - protein, 112 aa, Artificial Sequence
  19D7-IGKV3-15
EIVMTQSPATLSVSPGERATLSCRSSKSLLHSNGNTYLYWYQQKPGQAPRLLIYRVSNLASGIPARFSGSGSGTEFTLTISSLQSEDFAVYYCMQHLEYPFTFGQGTKLEIK

SEQ ID NO: 55 - protein, 112 aa, Artificial Sequence
  19D7-IGKV2-18
DIVMTQTPPSLPVNPGEPASISCRSSKSLLHSNGNTYLYWYLQKPGQSPQLLIYRVSNLASGVPDRFSGSGSGSDFTLKISWVEAEDVGVYYCMQHLEYPFTFGQGTKLEIK

SEQ ID NO: 56 - protein, 112 aa, Artificial Sequence
  19D7-IGKV3-20
EIVLTQSPGTLSLSPGERATLSCRSSKSLLHSNGNTYLYWYQQKPGQAPRLLIYRVSNLASGIPDRFSGSGSGTDFTLTISRLEPEDFAVYYCMQHLEYPFTFGQGTKLEIK

SEQ ID NO: 57 - protein, 123 aa, Artificial Sequence
  19D7-IGHV3-15 T94R
EVQLVESGGALVKPGGSLRLSCAASGFTFSTYAMYWVRQAPGKGLEWVGRIRSKSNNYATYYADSVKDRFTISRDDSKNTLYLQMNSLKTEDTAVYYCTRGGYGNYRYAMDYWGQGTTVTVSS

SEQ ID NO: 58 - protein, 123 aa, Artificial Sequence
  19D7-IGHV3-73
EVQLVESGGGLVQPGGSLKLSCAASGFTFSTYAMYWVRQASGKGLEWVGRIRSKSNNYATYYADSVKDRFTISRDDSKNTAYLQMNSLKTEDTAVYYCTRGGYGNYRYAMDYWGQGTTVTVSS

SEQ ID NO: 59 - protein, 114 aa, Artificial Sequence
  10A11-IGKV4-1 N53Q+G29R
DIVMTQSPDSLAVSLGERATINCRSSKSLLHSNRNTYLYWYQQKPGQPPKLLIYRMSQLASGVPDRFSGSGSGTDFTLTISSLQAEDVAVYYCMQHLEYPLTFGQGTKLEIKRT

SEQ ID NO: 60 - protein, 123 aa, Artificial Sequence
  19D7-IGHV3-15 K64R+T94R
EVQLVESGGALVKPGGSLRLSCAASGFTFSTYAMYWVRQAPGKGLEWVGRIRSKSNNYATYYADSVRDRFTISRDDSKNTLYLQMNSLKTEDTAVYYCTRGGYGNYRYAMDYWGQGTTVTVSS